European Patent Application EP 4 190 896 A1, published June 7, 2023. Title: COMPOSITIONS AND METHODS FOR ORDERED AND CONTINUOUS COMPLEMENTARY DNA (cDNA) SYNTHESIS ACROSS NON-CONTINUOUS TEMPLATES. Applicant: The Regents of the University of California. The sequence listing filed with the application follows.

SEQUENCE LISTING (23 sequences)

SEQ ID NO: 1 - protein, 1114 aa, Bombyx mori
MMASTALSLMGRCNPDGCTRGKHVTAAPMDGPRGPSSLAGTFGWGLAIPAGEPCGRVCSPATVGFFPVAKKSNKENRPEASGLPLESERTGDNPTVRGSAGADPVGQDAPGWTCQFCERTFSTNRGLGVHKRRAHPVETNTDAAPMMVKRRWHGEEIDLLARTEARLLAERGQCSGGDLFGALPGFGRTLEAIKGQRRREPYRALVQAHLARFGSQPGPSSGGCSAEPDFRRASGAEEAGEERCAEDAAAYDPSAVGQMSPDAARVLSELLEGAGRRRACRAMRPKTAGRRNDLHDDRTASAHKTSRQKRRAEYARVQELYKKCRSRAAAEVIDGACGGVGHSLEEMETYWRPILERVSDAPGPTPEALHALGRAEWHGGNRDYTQLWKPISVEEIKASRFDWRTSPGPDGIRSGQWRAVPVHLKAEMFNAWMARGEIPEILRQCRTVFVPKVERPGGPGEYRPISIASIPLRHFHSILARRLLACCPPDARQRGFICADGTLENSAVLDAVLGDSRKKLRECHVAVLDFAKAFDTVSHEALVELLRLRGMPEQFCGYIAHLYDTASTTLAVNNEMSSPVKVGRGVRQGDPLSPILFNVVMDLILASLPERVGYRLEMELVSALAYADDLVLLAGSKVGMQESISAVDCVGRQMGLRLNCRKSAVLSMIPDGHRKKHHYLTERTFNIGGKPLRQVSCVERWRYLGVDFEASGCVTLEHSISSALNNISRAPLKPQQRLEILRAHLIPRFQHGFVLGNISDDRLRMLDVQIRKAVGQWLRLPADVPKAYYHAAVQDGGLAIPSVRATIPDLIVRRFGGLDSSPWSVARAAAKSDKIRKKLRWAWKQLRRFSRVDSTTQRPSVRLFWREHLHASVDGRELRESTRTPTSTKWIRERCAQITGRDFVQFVHTHINALPSRIRGSRGRRGGGESSLTCRAGCKVRETTAHILQQCHRTHGGRILRHNKIVSFVAKAMEENKWTVELEPRLRTSVGLRKPDIIASRDGVGVIVDVQVVSGQRSLDELHREKRNKYGNHGELVELVAGRLGLPKAECVRATSCTISWRGVWSLTSYKELRSIIGLREPTLQIVPILALRGSHMNWTRFNQMTSVMGGGVG

SEQ ID NO: 2 - protein, 840 aa, synthetic construct
  REGION 1..840: note = Synthetic Construct
GRRRACRAMRPKTAGRRNDLHDDRTASAHKTSRQKRRAEYARVQELYKKCRSRAAAEVIDGACGGVGHSLEEMETYWRPILERVSDAPGPTPEALHALGRAEWHGGNRDYTQLWKPISVEEIKASRFDWRTSPGPDGIRSGQWRAVPVHLKAEMFNAWMARGEIPEILRQCRTVFVPKVERPGGPGEYRPISIASIPLRHFHSILARRLLACCPPDARQRGFICADGTLENSAVLDAVLGDSRKKLRECHVAVLDFAKAFDTVSHEALVELLRLRGMPEQFCGYIAHLYDTASTTLAVNNEMSSPVKVGRGVRQGDPLSPILFNVVMDLILASLPERVGYRLEMELVSALAYADDLVLLAGSKVGMQESISAVDCVGRQMGLRLNCRKSAVLSMIPDGHRKKHHYLTERTFNIGGKPLRQVSCVERWRYLGVDFEASGCVTLEHSISSALNNISRAPLKPQQRLEILRAHLIPRFQHGFVLGNISDDRLRMLDVQIRKAVGQWLRLPADVPKAYYHAAVQDGGLAIPSVRATIPDLIVRRFGGLDSSPWSVARAAAKSDKIRKKLRWAWKQLRRFSRVDSTTQRPSVRLFWREHLHASVDGRELRESTRTPTSTKWIRERCAQITGRDFVQFVHTHINALPSRIRGSRGRRGGGESSLTCRAGCKVRETTAHILQQCHRTHGGRILRHNKIVSFVAKAMEENKWTVELEPRLRTSVGLRKPAIIASRDGVGVIVDVQVVSGQRSLDELHREKRNKYGNHGELVELVAGRLGLPKAECVRATSCTISWRGVWSLTSYKELRSIIGLREPTLQIVPILALRGSHMNWTRFNQMTSVMGGGVG

SEQ ID NO: 3 - protein, 1228 aa, synthetic construct
  REGION 1..1228: note = Synthetic Construct
MKIEEGKLVIWINGDKGYNGLAEVGKKFEKDTGIKVTVEHPDKLEEKFPQVAATGDGPDIIFWAHDRFGGYAQSGLLAEITPDKAFQDKLYPFTWDAVRYNGKLIAYPIAVEALSLIYNKDLLPNPPKTWEEIPALDKELKAKGKSALMFNLQEPYFTWPLIAADGGYAFKYENGKYDIKDVGVDNAGAKAGLTFLVDLIKNKHMNADTDYSIAEAAFNKGETAMTINGPWAWSNIDTSKVNYGVTVLPTFKGQPSKPFVGVLSAGINAASPNKELAKEFLENYLLTDEGLEAVNKDKPLGAVALKSYEEELVKDPRIAATMENAQKGEIMPNIPQMSAFWYAVRTAVINAASGRQTVDEALAAAQTAAAAAMGRRRACRAMRPKTAGRRNDLHDDRTASAHKTSRQKRRAEYARVQELYKKCRSRAAAEVIDGACGGVGHSLEEMETYWRPILERVSDAPGPTPEALHALGRAEWHGGNRDYTQLWKPISVEEIKASRFDWRTSPGPDGIRSGQWRAVPVHLKAEMFNAWMARGEIPEILRQCRTVFVPKVERPGGPGEYRPISIASIPLRHFHSILARRLLACCPPDARQRGFICADGTLENSAVLDAVLGDSRKKLRECHVAVLDFAKAFDTVSHEALVELLRLRGMPEQFCGYIAHLYDTASTTLAVNNEMSSPVKVGRGVRQGDPLSPILFNVVMDLILASLPERVGYRLEMELVSALAYADDLVLLAGSKVGMQESISAVDCVGRQMGLRLNCRKSAVLSMIPDGHRKKHHYLTERTFNIGGKPLRQVSCVERWRYLGVDFEASGCVTLEHSISSALNNISRAPLKPQQRLEILRAHLIPRFQHGFVLGNISDDRLRMLDVQIRKAVGQWLRLPADVPKAYYHAAVQDGGLAIPSVRATIPDLIVRRFGGLDSSPWSVARAAAKSDKIRKKLRWAWKQLRRFSRVDSTTQRPSVRLFWREHLHASVDGRELRESTRTPTSTKWIRERCAQITGRDFVQFVHTHINALPSRIRGSRGRRGGGESSLTCRAGCKVRETTAHILQQCHRTHGGRILRHNKIVSFVAKAMEENKWTVELEPRLRTSVGLRKPAIIASRDGVGVIVDVQVVSGQRSLDELHREKRNKYGNHGELVELVAGRLGLPKAECVRATSCTISWRGVWSLTSYKELRSIIGLREPTLQIVPILALRGSHMNWTRFNQMTSVMGGGVGENLYFQSGSHHHHHH

SEQ ID NO: 4 - protein, 427 aa, Eubacterium rectale
MDTSNLMEQILSSDNLNRAYLQVVRNKGAEGVDGMKYTELKEHLAKNGETIKGQLRTRKYKPQPARRVEIPKPDGGVRNLGVPTVTDRFIQQAIAQVLTPIYEEQFHDHSYGFRPNRCAQQAILTALNIMNDGNDWIVDIDLEKFFDTVNHDKLMTLIGRTIKDGDVISIVRKYLVSGIMIDDEYEDSIVGTPQGGNLSPLLANIMLNELDKEMEKRGLNFVRYADDCIIMVGSEMSANRVMRNISRFIEEKLGLKVNMTKSKVDRPSGLKYLGFGFYFDPRAHQFKAKPHAKSVAKFKKRMKELTCRSWGVSNSYKVEKLNQLIRGWINYFKIGSMKTLCKELDSRIRYRLRMCIWKQWKTPQNQEKNLVKLGIDRNTARRVAYTGKRIAYVCNKGAVNVAISNKRLASFGLISMLDYYIEKCVTC

SEQ ID NO: 5 - protein, 1501 aa, synthetic construct
  REGION 1..1501: note = Synthetic Construct
MKIEEGKLVIWINGDKGYNGLAEVGKKFEKDTGIKVTVEHPDKLEEKFPQVAATGDGPDIIFWAHDRFGGYAQSGLLAEITPDKAFQDKLYPFTWDAVRYNGKLIAYPIAVEALSLIYNKDLLPNPPKTWEEIPALDKELKAKGKSALMFNLQEPYFTWPLIAADGGYAFKYENGKYDIKDVGVDNAGAKAGLTFLVDLIKNKHMNADTDYSIAEAAFNKGETAMTINGPWAWSNIDTSKVNYGVTVLPTFKGQPSKPFVGVLSAGINAASPNKELAKEFLENYLLTDEGLEAVNKDKPLGAVALKSYEEELVKDPRIAATMENAQKGEIMPNIPQMSAFWYAVRTAVINAASGRQTVDEALAAAQTAAAAAMMASTALSLMGRCNPDGCTRGKHVTAAPMDGPRGPSSLAGTFGWGLAIPAGEPCGRVCSPATVGFFPVAKKSNKENRPEASGLPLESERTGDNPTVRGSAGADPVGQDAPGWTCQFCERTFSTNRGLGVHKRRAHPVETNTDAAPMMVKRRWHGEEIDLLARTEARLLAERGQCSGGDLFGALPGFGRTLEAIKGQRRREPYRALVQAHLARFGSQPGPSSGGCSAEPDFRRASGAEEAGEERCAEDAAAYDPSAVGQMSPDAARVLSELLEGAGRRRACRAMRPKTAGRRNDLHDDRTASAHKTSRQKRRAEYARVQELYKKCRSRAAAEVIDGACGGVGHSLEEMETYWRPILERVSDAPGPTPEALHALGRAEWHGGNRDYTQLWKPISVEEIKASRFDWRTSPGPDGIRSGQWRAVPVHLKAEMFNAWMARGEIPEILRQCRTVFVPKVERPGGPGEYRPISIASIPLRHFHSILARRLLACCPPDARQRGFICADGTLENSAVLDAVLGDSRKKLRECHVAVLDFAKAFDTVSHEALVELLRLRGMPEQFCGYIAHLYDTASTTLAVNNEMSSPVKVGRGVRQGDPLSPILFNVVMDLILASLPERVGYRLEMELVSALAYADDLVLLAGSKVGMQESISAVDCVGRQMGLRLNCRKSAVLSMIPDGHRKKHHYLTERTFNIGGKPLRQVSCVERWRYLGVDFEASGCVTLEHSISSALNNISRAPLKPQQRLEILRAHLIPRFQHGFVLGNISDDRLRMLDVQIRKAVGQWLRLPADVPKAYYHAAVQDGGLAIPSVRATIPDLIVRRFGGLDSSPWSVARAAAKSDKIRKKLRWAWKQLRRFSRVDSTTQRPSVRLFWREHLHASVDGRELRESTRTPTSTKWIRERCAQITGRDFVQFVHTHINALPSRIRGSRGRRGGGESSLTCRAGCKVRETTAHILQQCHRTHGGRILRHNKIVSFVAKAMEENKWTVELEPRLRTSVGLRKPDIIASRDGVGVIVDVQVVSGQRSLDELHREKRNKYGNHGELVELVAGRLGLPKAECVRATSCTISWRGVWSLTSYKELRSIIGLREPTLQIVPILALRGSHMNWTRFNQMTSVMGGGVGENLYFQSGSHHHHHH

SEQ ID NO: 6 - protein, 1433 aa, synthetic construct
  REGION 1..1433: note = Synthetic Construct
MKIEEGKLVIWINGDKGYNGLAEVGKKFEKDTGIKVTVEHPDKLEEKFPQVAATGDGPDIIFWAHDRFGGYAQSGLLAEITPDKAFQDKLYPFTWDAVRYNGKLIAYPIAVEALSLIYNKDLLPNPPKTWEEIPALDKELKAKGKSALMFNLQEPYFTWPLIAADGGYAFKYENGKYDIKDVGVDNAGAKAGLTFLVDLIKNKHMNADTDYSIAEAAFNKGETAMTINGPWAWSNIDTSKVNYGVTVLPTFKGQPSKPFVGVLSAGINAASPNKELAKEFLENYLLTDEGLEAVNKDKPLGAVALKSYEEELVKDPRIAATMENAQKGEIMPNIPQMSAFWYAVRTAVINAASGRQTVDEALAAAQTAAAAAMKKSNKENRPEASGLPLESERTGDNPTVRGSAGADPVGQDAPGWTCQFCERTFSTNRGLGVHKRRAHPVETNTDAAPMMVKRRWHGEEIDLLARTEARLLAERGQCSGGDLFGALPGFGRTLEAIKGQRRREPYRALVQAHLARFGSQPGPSSGGCSAEPDFRRASGAEEAGEERCAEDAAAYDPSAVGQMSPDAARVLSELLEGAGRRRACRAMRPKTAGRRNDLHDDRTASAHKTSRQKRRAEYARVQELYKKCRSRAAAEVIDGACGGVGHSLEEMETYWRPILERVSDAPGPTPEALHALGRAEWHGGNRDYTQLWKPISVEEIKASRFDWRTSPGPDGIRSGQWRAVPVHLKAEMFNAWMARGEIPEILRQCRTVFVPKVERPGGPGEYRPISIASIPLRHFHSILARRLLACCPPDARQRGFICADGTLENSAVLDAVLGDSRKKLRECHVAVLDFAKAFDTVSHEALVELLRLRGMPEQFCGYIAHLYDTASTTLAVNNEMSSPVKVGRGVRQGDPLSPILFNVVMDLILASLPERVGYRLEMELVSALAYADDLVLLAGSKVGMQESISAVDCVGRQMGLRLNCRKSAVLSMIPDGHRKKHHYLTERTFNIGGKPLRQVSCVERWRYLGVDFEASGCVTLEHSISSALNNISRAPLKPQQRLEILRAHLIPRFQHGFVLGNISDDRLRMLDVQIRKAVGQWLRLPADVPKAYYHAAVQDGGLAIPSVRATIPDLIVRRFGGLDSSPWSVARAAAKSDKIRKKLRWAWKQLRRFSRVDSTTQRPSVRLFWREHLHASVDGRELRESTRTPTSTKWIRERCAQITGRDFVQFVHTHINALPSRIRGSRGRRGGGESSLTCRAGCKVRETTAHILQQCHRTHGGRILRHNKIVSFVAKAMEENKWTVELEPRLRTSVGLRKPDIIASRDGVGVIVDVQVVSGQRSLDELHREKRNKYGNHGELVELVAGRLGLPKAECVRATSCTISWRGVWSLTSYKELRSIIGLREPTLQIVPILALRGSHMNWTRFNQMTSVMGGGVGENLYFQSGSHHHHHH

SEQ ID NO: 7 - protein, 1228 aa, synthetic construct
  REGION 1..1228: note = Synthetic Construct
MKIEEGKLVIWINGDKGYNGLAEVGKKFEKDTGIKVTVEHPDKLEEKFPQVAATGDGPDIIFWAHDRFGGYAQSGLLAEITPDKAFQDKLYPFTWDAVRYNGKLIAYPIAVEALSLIYNKDLLPNPPKTWEEIPALDKELKAKGKSALMFNLQEPYFTWPLIAADGGYAFKYENGKYDIKDVGVDNAGAKAGLTFLVDLIKNKHMNADTDYSIAEAAFNKGETAMTINGPWAWSNIDTSKVNYGVTVLPTFKGQPSKPFVGVLSAGINAASPNKELAKEFLENYLLTDEGLEAVNKDKPLGAVALKSYEEELVKDPRIAATMENAQKGEIMPNIPQMSAFWYAVRTAVINAASGRQTVDEALAAAQTAAAAAMGRRRACRAMRPKTAGRRNDLHDDRTASAHKTSRQKRRAEYARVQELYKKCRSRAAAEVIDGACGGVGHSLEEMETYWRPILERVSDAPGPTPEALHALGRAEWHGGNRDYTQLWKPISVEEIKASRFDWRTSPGPDGIRSGQWRAVPVHLKAEMFNAWMARGEIPEILRQCRTVFVPKVERPGGPGEYRPISIASIPLRHFHSILARRLLACCPPDARQRGFICADGTLENSAVLDAVLGDSRKKLRECHVAVLDFAKAFDTVSHEALVELLRLRGMPEQFCGYIAHLYDTASTTLAVNNEMSSPVKVGRGVRQGDPLSPILFNVVMDLILASLPERVGYRLEMELVSALAYADDLVLLAGSKVGMQESISAVDCVGRQMGLRLNCRKSAVLSMIPDGHRKKHHYLTERTFNIGGKPLRQVSCVERWRYLGVDFEASGCVTLEHSISSALNNISRAPLKPQQRLEILRAHLIPRFQHGFVLGNISDDRLRMLDVQIRKAVGQWLRLPADVPKAYYHAAVQDGGLAIPSVRATIPDLIVRRFGGLDSSPWSVARAAAKSDKIRKKLRWAWKQLRRFSRVDSTTQRPSVRLFWREHLHASVDGRELRESTRTPTSTKWIRERCAQITGRDFVQFVHTHINALPSRIRGSRGRRGGGESSLTCRAGCKVRETTAHILQQCHRTHGGRILRHNKIVSFVAKAMEENKWTVELEPRLRTSVGLRKPDIIASRDGVGVIVDVQVVSGQRSLDELHREKRNKYGNHGELVELVAGRLGLPKAECVRATSCTISWRGVWSLTSYKELRSIIGLREPTLQIVPILALRGSHMNWTRFNQMTSVMGGGVGENLYFQSGSHHHHHH

SEQ ID NO: 8 - protein, 814 aa, synthetic construct
  REGION 1..814: note = Synthetic Construct
MKIEEGKLVIWINGDKGYNGLAEVGKKFEKDTGIKVTVEHPDKLEEKFPQVAATGDGPDIIFWAHDRFGGYAQSGLLAEITPDKAFQDKLYPFTWDAVRYNGKLIAYPIAVEALSLIYNKDLLPNPPKTWEEIPALDKELKAKGKSALMFNLQEPYFTWPLIAADGGYAFKYENGKYDIKDVGVDNAGAKAGLTFLVDLIKNKHMNADTDYSIAEAAFNKGETAMTINGPWAWSNIDTSKVNYGVTVLPTFKGQPSKPFVGVLSAGINAASPNKELAKEFLENYLLTDEGLEAVNKDKPLGAVALKSYEEELVKDPRIAATMENAQKGEIMPNIPQMSAFWYAVRTAVINAASGRQTVDEALAAAQTAAAAAMDTSNLMEQILSSDNLNRAYLQVVRNKGAEGVDGMKYTELKEHLAKNGETIKGQLRTRKYKPQPARRVEIPKPDGGVRNLGVPTVTDRFIQQAIAQVLTPIYEEQFHDHSYGFRPNRCAQQAILTALNIMNDGNDWIVDIDLEKFFDTVNHDKLMTLIGRTIKDGDVISIVRKYLVSGIMIDDEYEDSIVGTPQGGNLSPLLANIMLNELDKEMEKRGLNFVRYADDCIIMVGSEMSANRVMRNISRFIEEKLGLKVNMTKSKVDRPSGLKYLGFGFYFDPRAHQFKAKPHAKSVAKFKKRMKELTCRSWGVSNSYKVEKLNQLIRGWINYFKIGSMKTLCKELDSRIRYRLRMCIWKQWKTPQNQEKNLVKLGIDRNTARRVAYTGKRIAYVCNKGAVNVAISNKRLASFGLISMLDYYIEKCVTCENLYFQSGSHHHHHH

SEQ ID NO: 9 - protein, 1045 aa, Bombyx mori
KKSNKENRPEASGLPLESERTGDNPTVRGSAGADPVGQDAPGWTCQFCERTFSTNRGLGVHKRRAHPVETNTDAAPMMVKRRWHGEEIDLLARTEARLLAERGQCSGGDLFGALPGFGRTLEAIKGQRRREPYRALVQAHLARFGSQPGPSSGGCSAEPDFRRASGAEEAGEERCAEDAAAYDPSAVGQMSPDAARVLSELLEGAGRRRACRAMRPKTAGRRNDLHDDRTASAHKTSRQKRRAEYARVQELYKKCRSRAAAEVIDGACGGVGHSLEEMETYWRPILERVSDAPGPTPEALHALGRAEWHGGNRDYTQLWKPISVEEIKASRFDWRTSPGPDGIRSGQWRAVPVHLKAEMFNAWMARGEIPEILRQCRTVFVPKVERPGGPGEYRPISIASIPLRHFHSILARRLLACCPPDARQRGFICADGTLENSAVLDAVLGDSRKKLRECHVAVLDFAKAFDTVSHEALVELLRLRGMPEQFCGYIAHLYDTASTTLAVNNEMSSPVKVGRGVRQGDPLSPILFNVVMDLILASLPERVGYRLEMELVSALAYADDLVLLAGSKVGMQESISAVDCVGRQMGLRLNCRKSAVLSMIPDGHRKKHHYLTERTFNIGGKPLRQVSCVERWRYLGVDFEASGCVTLEHSISSALNNISRAPLKPQQRLEILRAHLIPRFQHGFVLGNISDDRLRMLDVQIRKAVGQWLRLPADVPKAYYHAAVQDGGLAIPSVRATIPDLIVRRFGGLDSSPWSVARAAAKSDKIRKKLRWAWKQLRRFSRVDSTTQRPSVRLFWREHLHASVDGRELRESTRTPTSTKWIRERCAQITGRDFVQFVHTHINALPSRIRGSRGRRGGGESSLTCRAGCKVRETTAHILQQCHRTHGGRILRHNKIVSFVAKAMEENKWTVELEPRLRTSVGLRKPDIIASRDGVGVIVDVQVVSGQRSLDELHREKRNKYGNHGELVELVAGRLGLPKAECVRATSCTISWRGVWSLTSYKELRSIIGLREPTLQIVPILALRGSHMNWTRFNQMTSVMGGGVG

SEQ ID NO: 10 - protein, 840 aa, Bombyx mori
GRRRACRAMRPKTAGRRNDLHDDRTASAHKTSRQKRRAEYARVQELYKKCRSRAAAEVIDGACGGVGHSLEEMETYWRPILERVSDAPGPTPEALHALGRAEWHGGNRDYTQLWKPISVEEIKASRFDWRTSPGPDGIRSGQWRAVPVHLKAEMFNAWMARGEIPEILRQCRTVFVPKVERPGGPGEYRPISIASIPLRHFHSILARRLLACCPPDARQRGFICADGTLENSAVLDAVLGDSRKKLRECHVAVLDFAKAFDTVSHEALVELLRLRGMPEQFCGYIAHLYDTASTTLAVNNEMSSPVKVGRGVRQGDPLSPILFNVVMDLILASLPERVGYRLEMELVSALAYADDLVLLAGSKVGMQESISAVDCVGRQMGLRLNCRKSAVLSMIPDGHRKKHHYLTERTFNIGGKPLRQVSCVERWRYLGVDFEASGCVTLEHSISSALNNISRAPLKPQQRLEILRAHLIPRFQHGFVLGNISDDRLRMLDVQIRKAVGQWLRLPADVPKAYYHAAVQDGGLAIPSVRATIPDLIVRRFGGLDSSPWSVARAAAKSDKIRKKLRWAWKQLRRFSRVDSTTQRPSVRLFWREHLHASVDGRELRESTRTPTSTKWIRERCAQITGRDFVQFVHTHINALPSRIRGSRGRRGGGESSLTCRAGCKVRETTAHILQQCHRTHGGRILRHNKIVSFVAKAMEENKWTVELEPRLRTSVGLRKPDIIASRDGVGVIVDVQVVSGQRSLDELHREKRNKYGNHGELVELVAGRLGLPKAECVRATSCTISWRGVWSLTSYKELRSIIGLREPTLQIVPILALRGSHMNWTRFNQMTSVMGGGVG

SEQ ID NO: 11 - protein, 811 aa, synthetic construct
  REGION 1..811: note = Synthetic Construct
KTSRQKRRAEYARVQELYKKCRSRAAAEVIDGACGGVGHSLEEMETYWRPILERVSDAPGPTPEALHALGRAEWHGGNRDYTQLWKPISVEEIKASRFDWRTSPGPDGIRSGQWRAVPVHLKAEMFNAWMARGEIPEILRQCRTVFVPKVERPGGPGEYRPISIASIPLRHFHSILARRLLACCPPDARQRGFICADGTLENSAVLDAVLGDSRKKLRECHVAVLDFAKAFDTVSHEALVELLRLRGMPEQFCGYIAHLYDTASTTLAVNNEMSSPVKVGRGVRQGDPLSPILFNVVMDLILASLPERVGYRLEMELVSALAYADDLVLLAGSKVGMQESISAVDCVGRQMGLRLNCRKSAVLSMIPDGHRKKHHYLTERTFNIGGKPLRQVSCVERWRYLGVDFEASGCVTLEHSISSALNNISRAPLKPQQRLEILRAHLIPRFQHGFVLGNISDDRLRMLDVQIRKAVGQWLRLPADVPKAYYHAAVQDGGLAIPSVRATIPDLIVRRFGGLDSSPWSVARAAAKSDKIRKKLRWAWKQLRRFSRVDSTTQRPSVRLFWREHLHASVDGRELRESTRTPTSTKWIRERCAQITGRDFVQFVHTHINALPSRIRGSRGRRGGGESSLTCRAGCKVRETTAHILQQCHRTHGGRILRHNKIVSFVAKAMEENKWTVELEPRLRTSVGLRKPAIIASRDGVGVIVDVQVVSGQRSLDELHREKRNKYGNHGELVELVAGRLGLPKAECVRATSCTISWRGVWSLTSYKELRSIIGLREPTLQIVPILALRGSHMNWTRFNQMTSVMGGGVG

SEQ ID NO: 12 - protein, 1199 aa, synthetic construct
  REGION 1..1199: note = Synthetic Construct
MKIEEGKLVIWINGDKGYNGLAEVGKKFEKDTGIKVTVEHPDKLEEKFPQVAATGDGPDIIFWAHDRFGGYAQSGLLAEITPDKAFQDKLYPFTWDAVRYNGKLIAYPIAVEALSLIYNKDLLPNPPKTWEEIPALDKELKAKGKSALMFNLQEPYFTWPLIAADGGYAFKYENGKYDIKDVGVDNAGAKAGLTFLVDLIKNKHMNADTDYSIAEAAFNKGETAMTINGPWAWSNIDTSKVNYGVTVLPTFKGQPSKPFVGVLSAGINAASPNKELAKEFLENYLLTDEGLEAVNKDKPLGAVALKSYEEELVKDPRIAATMENAQKGEIMPNIPQMSAFWYAVRTAVINAASGRQTVDEALAAAQTAAAAAMKTSRQKRRAEYARVQELYKKCRSRAAAEVIDGACGGVGHSLEEMETYWRPILERVSDAPGPTPEALHALGRAEWHGGNRDYTQLWKPISVEEIKASRFDWRTSPGPDGIRSGQWRAVPVHLKAEMFNAWMARGEIPEILRQCRTVFVPKVERPGGPGEYRPILIASIPLRHFHSILARRLLACCPPDARQRGFICADGTLENSAVLDAVLGDSRKKLRECHVAVLDFAKAFDTVSHEALVELLRLRGMPEQFCGYIAHLYDTASTTLAVNNEMSSPVKVGRGVRQGDPLSPILFNVVMDLILASLPERVGYRLEMELVSALAYADDLVLLAGSKVGMQESISAVDCVGKQMGLRLNCRKSAVLSMIPDGHRKKHHYLTERTFNIGGKPLRQVSCVERWRYLGVDFEASGCVTLEHSISSALNNISRAPLKPQQRLEILRAHLIPRFQHGFVLGNISDDRLRMLDVQIRKAVGQWLRLPADVPKAYYHAAVQDGGLAIPSVRATIPDLIVRRFGGLDSSPWSVARAAAKSDKIRKKLRWAWKQLRRFSRVDSTTQRPSVRLFWREHLHASVDGRELRESTRTPTSTKWIRERCAQITGRDFVQFVHTHINALPSRIRGSRGRRGGGESSLTCRAGCKVRETTAHILQQCHRTHGGRILRHNKIVSFVAKAMEENKWTVELEPRLRTSVGLRKPAIIASRDGVGVIVDVQVVSGQRSLDELHREKRNKYGNHGELVELVAGRLGLPKAECVRATSCTISWRGVWSLTSYKELRSIIGLREPTLQIVPILALRGSHMNWTRFNQMTSVMGGGVGENLYFQSGSHHHHHH

SEQ ID NO: 13 - protein, 1433 aa, synthetic construct
  REGION 1..1433: note = Synthetic Construct
MKIEEGKLVIWINGDKGYNGLAEVGKKFEKDTGIKVTVEHPDKLEEKFPQVAATGDGPDIIFWAHDRFGGYAQSGLLAEITPDKAFQDKLYPFTWDAVRYNGKLIAYPIAVEALSLIYNKDLLPNPPKTWEEIPALDKELKAKGKSALMFNLQEPYFTWPLIAADGGYAFKYENGKYDIKDVGVDNAGAKAGLTFLVDLIKNKHMNADTDYSIAEAAFNKGETAMTINGPWAWSNIDTSKVNYGVTVLPTFKGQPSKPFVGVLSAGINAASPNKELAKEFLENYLLTDEGLEAVNKDKPLGAVALKSYEEELVKDPRIAATMENAQKGEIMPNIPQMSAFWYAVRTAVINAASGRQTVDEALAAAQTAAAAAMKKSNKENRPEASGLPLESERTGDNPTVRGSAGADPVGQDAPGWTCQFCERTFSTNRGLGVHKRRAHPVETNTDAAPMMVKRRWHGEEIDLLARTEARLLAERGQCSGGDLFGALPGFGRTLEAIKGQRRREPYRALVQAHLARFGSQPGPSSGGCSAEPDFRRASGAEEAGEERCAEDAAAYDPSAVGQMSPDAARVLSELLEGAGRRRACRAMRPKTAGRRNDLHDDRTASAHKTSRQKRRAEYARVQELYKKCRSRAAAEVIDGACGGVGHSLEEMETYWRPILERVSDAPGPTPEALHALGRAEWHGGNRDYTQLWKPISVEEIKASRFDWRTSPGPDGIRSGQWRAVPVHLKAEMFNAWMARGEIPEILRQCRTVFVPKVERPGGPGEYRPISIASIPLRHFHSILARRLLACCPPDARQRGFICADGTLENSAVLDAVLGDSRKKLRECHVAVLDFAKAFDTVSHEALVELLRLRGMPEQFCGYIAHLYDTASTTLAVNNEMSSPVKVGRGVRQGDPLSPILFNVVMDLILASLPERVGYRLEMELVSALAYADDLVLLAGSKVGMQESISAVDCVGRQMGLRLNCRKSAVLSMIPDGHRKKHHYLTERTFNIGGKPLRQVSCVERWRYLGVDFEASGCVTLEHSISSALNNISRAPLKPQQRLEILRAHLIPRFQHGFVLGNISDDRLRMLDVQIRKAVGQWLRLPADVPKAYYHAAVQDGGLAIPSVRATIPDLIVRRFGGLDSSPWSVARAAAKSDKIRKKLRWAWKQLRRFSRVDSTTQRPSVRLFWREHLHASVDGRELRESTRTPTSTKWIRERCAQITGRDFVQFVHTHINALPSRIRGSRGRRGGGESSLTCRAGCKVRETTAHILQQCHRTHGGRILRHNKIVSFVAKAMEENKWTVELEPRLRTSVGLRKPAIIASRDGVGVIVDVQVVSGQRSLDELHREKRNKYGNHGELVELVAGRLGLPKAECVRATSCTISWRGVWSLTSYKELRSIIGLREPTLQIVPILALRGSHMNWTRFNQMTSVMGGGVGENLYFQSGSHHHHHH

SEQ ID NO: 14 - protein, 1045 aa, synthetic construct
  REGION 1..1045: note = Synthetic Construct
KKSNKENRPEASGLPLESERTGDNPTVRGSAGADPVGQDAPGWTCQFCERTFSTNRGLGVHKRRAHPVETNTDAAPMMVKRRWHGEEIDLLARTEARLLAERGQCSGGDLFGALPGFGRTLEAIKGQRRREPYRALVQAHLARFGSQPGPSSGGCSAEPDFRRASGAEEAGEERCAEDAAAYDPSAVGQMSPDAARVLSELLEGAGRRRACRAMRPKTAGRRNDLHDDRTASAHKTSRQKRRAEYARVQELYKKCRSRAAAEVIDGACGGVGHSLEEMETYWRPILERVSDAPGPTPEALHALGRAEWHGGNRDYTQLWKPISVEEIKASRFDWRTSPGPDGIRSGQWRAVPVHLKAEMFNAWMARGEIPEILRQCRTVFVPKVERPGGPGEYRPISIASIPLRHFHSILARRLLACCPPDARQRGFICADGTLENSAVLDAVLGDSRKKLRECHVAVLDFAKAFDTVSHEALVELLRLRGMPEQFCGYIAHLYDTASTTLAVNNEMSSPVKVGRGVRQGDPLSPILFNVVMDLILASLPERVGYRLEMELVSALAYADDLVLLAGSKVGMQESISAVDCVGRQMGLRLNCRKSAVLSMIPDGHRKKHHYLTERTFNIGGKPLRQVSCVERWRYLGVDFEASGCVTLEHSISSALNNISRAPLKPQQRLEILRAHLIPRFQHGFVLGNISDDRLRMLDVQIRKAVGQWLRLPADVPKAYYHAAVQDGGLAIPSVRATIPDLIVRRFGGLDSSPWSVARAAAKSDKIRKKLRWAWKQLRRFSRVDSTTQRPSVRLFWREHLHASVDGRELRESTRTPTSTKWIRERCAQITGRDFVQFVHTHINALPSRIRGSRGRRGGGESSLTCRAGCKVRETTAHILQQCHRTHGGRILRHNKIVSFVAKAMEENKWTVELEPRLRTSVGLRKPAIIASRDGVGVIVDVQVVSGQRSLDELHREKRNKYGNHGELVELVAGRLGLPKAECVRATSCTISWRGVWSLTSYKELRSIIGLREPTLQIVPILALRGSHMNWTRFNQMTSVMGGGVG

SEQ ID NO: 15 - DNA, 66 bp, synthetic construct
  misc_feature 1..66: note = Synthetic Construct
  source 1..66: mol_type = other DNA
caagcagaagacggcatacgagatgacgagaggtgactggagttcagacgtgtgctcttccgatct

SEQ ID NO: 16 - RNA, 31 nt, synthetic construct
  misc_feature 1..31: note = Synthetic Construct
  misc_feature 31: note = N is a 3' C3 Spacer
  source 1..31: mol_type = other RNA
gatcggaagagcacacgtctgaactccagtn

SEQ ID NO: 17 - DNA, 72 bp, synthetic construct
  misc_feature 1..72: note = Synthetic Construct
  misc_feature 1: note = N is a 5' C6 amino modifier
  source 1..72: mol_type = other DNA
naatgatacggcgaccaccgagatctacaccgcagacgacactctttccctacacgacgctcttccgatctc

SEQ ID NO: 18 - RNA, 31 nt, synthetic construct
  misc_feature 1..31: note = Synthetic Construct
  misc_feature 1: note = N is a 5' C3 Spacer
  misc_feature 31: note = N is a 3' C3 Spacer
  source 1..31: mol_type = other RNA
ngtgtagatctcggtggtcgccgtatcattn

SEQ ID NO: 19 - DNA, 34 bp, synthetic construct
  misc_feature 1..34: note = Synthetic Construct
  source 1..34: mol_type = other DNA
gtgactggagttcagacgtgtgctcttccgatcc

SEQ ID NO: 20 - RNA, 31 nt, synthetic construct; identical to SEQ ID NO: 16
  misc_feature 1..31: note = Synthetic Construct
  misc_feature 31: note = N is a 3' C3 Spacer
  source 1..31: mol_type = other RNA

SEQ ID NO: 21 - DNA, 34 bp, synthetic construct
  misc_feature 1..34: note = Synthetic Construct
  modified_base 1: mod_base = OTHER; note = 5' Phosphorylation
  source 1..34: mol_type = other DNA
acactctttccctacacgacgctcttccgatctc

SEQ ID NO: 22 - DNA, 52 bp, synthetic construct
  misc_feature 1..52: note = Synthetic Construct
  source 1..52: mol_type = other DNA
caagcagaagacggcatacgagattcgatccagtgactggagttcagacgtg

SEQ ID NO: 23 - DNA, 57 bp, synthetic construct
  misc_feature 1..57: note = Synthetic Construct
  source 1..57: mol_type = other DNA
aatgatacggcgaccaccgagatctacaccgcagacgacactctttccctacacgac